European Patent Application EP 4 166 156 A1, published April 19, 2023. Title: Composition Comprising Pentapeptide as an Active Ingredient for the Prevention, Improvement or Treatment of Allergic Diseases or Itching. Applicant: CAREGEN CO., LTD. The sequence listing filed with the application follows.

SEQUENCE LISTING (13 sequences)

SEQ ID NO: 1 - protein, 5 aa, Artificial Sequence
  Pentapeptide
KFLIK

SEQ ID NO: 2 - DNA, 21 bp, Artificial Sequence
  Forward primer for IL-3
ccagatttcagacaggggctc

SEQ ID NO: 3 - DNA, 21 bp, Artificial Sequence
  Reverse primer for IL-3
caggtttactctccgcaaggt

SEQ ID NO: 4 - DNA, 20 bp, Artificial Sequence
  Forward primer for IL-4
tccacggatgtaacgacagc

SEQ ID NO: 5 - DNA, 20 bp, Artificial Sequence
  Reverse primer for IL-4
tcattcacggtgcagcttct

SEQ ID NO: 6 - DNA, 20 bp, Artificial Sequence
  Forward primer for TNF-alpha
atgggctccctctcatcagt

SEQ ID NO: 7 - DNA, 20 bp, Artificial Sequence
  Reverse primer for TNF-alpha
gaaatggcaaatcggctgac

SEQ ID NO: 8 - DNA, 21 bp, Artificial Sequence
  Forward primer for TNF-alpha
aacatccaaccttcccaaacg

SEQ ID NO: 9 - DNA, 21 bp, Artificial Sequence
  Reverse primer for TNF-alpha
gaccctaagcccccaattctc

SEQ ID NO: 10 - DNA, 20 bp, Artificial Sequence
  Forward primer for IL-1beta
tgagtggtagccagcaaagc

SEQ ID NO: 11 - DNA, 20 bp, Artificial Sequence
  Reverse primer for IL-1beta
ctgcagtccaggttcaatgg

SEQ ID NO: 12 - DNA, 20 bp, Artificial Sequence
  Forward primer for COX-2
ttcgacacatgggataacga

SEQ ID NO: 13 - DNA, 20 bp, Artificial Sequence
  Reverse primer for COX-2
tctttcaacacgcaggacag